European Patent Specification EP 3 555 129 B1, published May 6, 2026. Title: Gremlin-1 crystal structure and inhibitory antibody. Applicant: UCB Biopharma SPRL. The sequence listing filed with the application follows.

SEQUENCE LISTING (35 sequences)

SEQ ID NO: 1 - protein, 184 aa, Artificial Sequence
  recombinant sequence
MSRTAYTVGALLLLLGTLLPAAEGKKKGSQGAIPPPDKAQHNDSEQTQSPQQPGSRNRGRGQGRGTAMPGEEVLESSQEALHVTERKYLKRDWCKTQPLKQTIHEEGCNSRTIINRFCYGQCNSFYIPRHIRKEEGSFQSCSFCKPKKFTTMMVTLNCPELQPPTKKKRVTRVKQCRCISIDLD

SEQ ID NO: 2 - protein, 139 aa, Artificial Sequence
  recombinant sequence
MGSSHHHHHHSSGENLYFQGSAMPGEEVLESSQEALHVTERKYLKRDWCKTQPLKQTIHEEGCNSRTIINRFCYGQCNSFYIPRHIRKEEGSFQSCSFCKPKKFTTMMVTLNCPELQPPTKKKRVTRVKQCRCISIDLD

SEQ ID NO: 3 - protein, 10 aa, Artificial Sequence
  recombinant sequence
GYTFTDYYMH

SEQ ID NO: 4 - protein, 5 aa, Artificial Sequence
  recombinant sequence
DYYMH

SEQ ID NO: 5 - protein, 17 aa, Artificial Sequence
  recombinant sequence
LVDPEDGETIYAEKFQG

SEQ ID NO: 6 - protein, 15 aa, Artificial Sequence
  recombinant sequence
DARGSGSYYPNHFDY

SEQ ID NO: 7 - protein, 17 aa, Artificial Sequence
  recombinant sequence
KSSQSVLYSSNNKNYLA

SEQ ID NO: 8 - protein, 7 aa, Artificial Sequence
  recombinant sequence
WASTRES

SEQ ID NO: 9 - protein, 8 aa, Artificial Sequence
  recombinant sequence
QQYYDTPT

SEQ ID NO: 10 - protein, 124 aa, Artificial Sequence
  recombinant sequence
QVQLVESGAEVKKPGATVKISCKVSGYTFTDYYMHWVQQAPGKGLEWMGLVDPEDGETIYAEKFQGRVTITADTSTDTAYMELSSLRSEDTAVYYCATDARGSGSYYPNHFDYWGQGTLVTVSS

SEQ ID NO: 11 - protein, 112 aa, Artificial Sequence
  recombinant sequence
DIVMTQSPDSLAVSLGERATINCKSSQSVLYSSNNKNYLAWYQQKPGQPPKLLIYWASTRESGVPDRFSGSGSGTDFTLTINSLQAEDVAVYFCQQYYDTPTFGQGTRLEIK

SEQ ID NO: 12 - protein, 124 aa, Artificial Sequence
  recombinant sequence
QVQLVQSGAEVKKPGATVKISCKVSGYTFTDYYMHWVQQAPGKGLEWMGLVDPEDGETIYAEKFQGRVTITADTSTDTAYMELSSLRSEDTAVYYCATDARGSGSYYPNHFDYWGQGTLVTVSS

SEQ ID NO: 13 - protein, 112 aa, Artificial Sequence
  recombinant sequence
DIVMTQTPDSLAVSLGERATINCKSSQSVLYSSNNKNYLAWYQQKPGQPPKLLIYWASTRESGVPDRFSGSGSGTDFTLTINSLQAEDVAVYFCQQYYDTPTFGQGTRLEIK

SEQ ID NO: 14 - protein, 448 aa, Artificial Sequence
  recombinant sequence
QVQLVESGAEVKKPGATVKISCKVSGYTFTDYYMHWVQQAPGKGLEWMGLVDPEDGETIYAEKFQGRVTITADTSTDTAYMELSSLRSEDTAVYYCATDARGSGSYYPNHFDYWGQGTLVTVSSAKTTPPSVYPLAPGSAAQTNSMVTLGCLVKGYFPEPVTVTWNSGSLSSGVHTFPAVLQSDLYTLSSSVTVPSSTWPSETVTCNVAHPASSTKVDKKIVPRDCGCKPCICTVPEVSSVFIFPPKPKDVLTITLTPKVTCVVVDISKDDPEVQFSWFVDDVEVHTAQTQPREEQFNSTFRSVSELPIMHQDWLNGKEFKCRVNSAAFPAPIEKTISKTKGRPKAPQVYTIPPPKEQMAKDKVSLTCMITDFFPEDITVEWQWNGQPAENYKNTQPIMDTDGSYFVYSKLNVQKSNWEAGNTFTCSVLHEGLHNHHTEKSLSHSPGK

SEQ ID NO: 15 - protein, 219 aa, Artificial Sequence
  recombinant sequence
DIVMTQSPDSLAVSLGERATINCKSSQSVLYSSNNKNYLAWYQQKPGQPPKLLIYWASTRESGVPDRFSGSGSGTDFTLTINSLQAEDVAVYFCQQYYDTPTFGQGTRLEIKRTDAAPTVSIFPPSSEQLTSGGASVVCFLNNFYPKDINVKWKIDGSERQNGVLNSWTDQDSKDSTYSMSSTLTLTKDEYERHNSYTCEATHKTSTSPIVKSFNRNEC

SEQ ID NO: 16 - protein, 454 aa, Artificial Sequence
  recombinant sequence
QVQLVQSGAEVKKPGATVKISCKVSGYTFTDYYMHWVQQAPGKGLEWMGLVDPEDGETIYAEKFQGRVTITADTSTDTAYMELSSLRSEDTAVYYCATDARGSGSYYPNHFDYWGQGTLVTVSSASTKGPSVFPLAPSSKSTSGGTAALGCLVKDYFPEPVTVSWNSGALTSGVHTFPAVLQSSGLYSLSSVVTVPSSSLGTQTYICNVNHKPSNTKVDKKVEPKSCDKTHTCPPCPAPELLGGPSVFLFPPKPKDTLMISRTPEVTCVVVDVSHEDPEVKFNWYVDGVEVHNAKTKPREEQYNSTYRVVSVLTVLHQDWLNGKEYKCKVSNKALPAPIEKTISKAKGQPREPQVYTLPPSRDELTKNQVSLTCLVKGFYPSDIAVEWESNGQPENNYKTTPPVLDSDGSFFLYSKLTVDKSRWQQGNVFSCSVMHEALHNHYTQKSLSLSPGK

SEQ ID NO: 17 - protein, 219 aa, Artificial Sequence
  recombinant sequence
DIVMTQTPDSLAVSLGERATINCKSSQSVLYSSNNKNYLAWYQQKPGQPPKLLIYWASTRESGVPDRFSGSGSGTDFTLTINSLQAEDVAVYFCQQYYDTPTFGQGTRLEIKRTVAAPSVFIFPPSDEQLKSGTASVVCLLNNFYPREAKVQWKVDNALQSGNSQESVTEQDSKDSTYSLSSTLTLSKADYEKHKVYACEVTHQGLSSPVTKSFNRGEC

SEQ ID NO: 18 - protein, 227 aa, Artificial Sequence
  recombinant sequence
QVQLVESGAEVKKPGATVKISCKVSGYTFTDYYMHWVQQAPGKGLEWMGLVDPEDGETIYAEKFQGRVTITADTSTDTAYMELSSLRSEDTAVYYCATDARGSGSYYPNHFDYWGQGTLVTVSSASTKGPSVFPLAPSSKSTSGGTAALGCLVKDYFPEPVTVSWNSGALTSGVHTFPAVLQSSGLYSLSSVVTVPSSSLGTQTYICNVNHKPSNTKVDKKVEPKSC

SEQ ID NO: 19 - protein, 219 aa, Artificial Sequence
  recombinant sequence
DIVMTQSPDSLAVSLGERATINCKSSQSVLYSSNNKNYLAWYQQKPGQPPKLLIYWASTRESGVPDRFSGSGSGTDFTLTINSLQAEDVAVYFCQQYYDTPTFGQGTRLEIKRTVAAPSVFIFPPSDEQLKSGTASVVCLLNNFYPREAKVQWKVDNALQSGNSQESVTEQDSKDSTYSLSSTLTLSKADYEKHKVYACEVTHQGLSSPVTKSFNRGEC

SEQ ID NO: 20 - protein, 118 aa, Artificial Sequence
  recombinant sequence
AMPGEEVLESSQEALHVTERKYLKRDWCKTQPLKQTIHEEGCNSRTIINRFCYGQCNSFYIPRHIRKEEGSFQSCSFCKPKKFTTMMVTLNCPELQPPTKKKRVTRVKQCRCISIDLD

SEQ ID NO: 21 - protein, 160 aa, Artificial Sequence
  recombinant sequence
KKKGSQGAIPPPDKAQHNDSEQTQSPQQPGSRNRGRGQGRGTAMPGEEVLESSQEALHVTERKYLKRDWCKTQPLKQTIHEEGCNSRTIINRFCYGQCNSFYIPRHIRKEEGSFQSCSFCKPKKFTTMMVTLNCPELQPPTKKKRVTRVKQCRCISIDLD

SEQ ID NO: 22 - protein, 451 aa, Artificial Sequence
  recombinant sequence
QVQLVESGAEVKKPGATVKISCKVSGYTFTDYYMHWVQQAPGKGLEWMGLVDPEDGETIYAEKFQGRVTITADTSTDTAYMELSSLRSEDTAVYYCATDARGSGSYYPNHFDYWGQGTLVTVSSASTKGPSVFPLAPCSRSTSESTAALGCLVKDYFPEPVTVSWNSGALTSGVHTFPAVLQSSGLYSLSSVVTVPSSSLGTKTYTCNVDHKPSNTKVDKRVESKYGPPCPPCPAPEFLGGPSVFLFPPKPKDTLMISRTPEVTCVVVDVSQEDPEVQFNWYVDGVEVHNAKTKPREEQFNSTYRVVSVLTVLHQDWLNGKEYKCKVSNKGLPSSIEKTISKAKGQPREPQVYTLPPSQEEMTKNQVSLTCLVKGFYPSDIAVEWESNGQPENNYKTTPPVLDSDGSFFLYSRLTVDKSRWQEGNVFSCSVMHEALHNHYTQKSLSLSLGK

SEQ ID NO: 23 - protein, 219 aa, Artificial Sequence; identical to SEQ ID NO: 19
  recombinant sequence

SEQ ID NO: 24 - DNA, 1362 bp, Artificial Sequence
  recombinant sequence
caagtgcaactggtggaatccggggccgaagtgaaaaagcccggagccactgtgaagatctcttgcaaagtgtccggctacaccttcaccgactattacatgcactgggtccagcaggcacctgggaagggccttgagtggatgggtctggtcgatcccgaggacggcgaaactatctacgccgagaagttccagggtcgcgtcaccatcaccgccgacacttccaccgacaccgcgtacatggagctgtccagcttgaggtccgaggacacagccgtgtactactgcgccacggatgctcggggaagcggcagctactacccgaaccacttcgactactggggacagggcactctcgtgactgtctcgagcgcttctacaaagggcccctccgtgttcccgctcgctccatcatcgaagtctaccagcggaggcactgcggctctcggttgcctcgtgaaggactacttcccggagccggtgaccgtgtcgtggaacagcggagccctgaccagcggggtgcacacctttccggccgtcttgcagtcaagcggcctttactccctgtcatcagtggtgactgtcccgtccagctcattgggaacccaaacctacatctgcaatgtgaatcacaaacctagcaacaccaaggttgacaagaaagtcgagcccaaatcgtgtgacaagactcacacttgtccgccgtgcccggcacccgaactgctgggaggtcccagcgtctttctgttccctccaaagccgaaagacacgctgatgatctcccgcaccccggaggtcacttgcgtggtcgtggacgtgtcacatgaggacccagaggtgaagttcaattggtacgtggatggcgtcgaagtccacaatgccaaaactaagcccagagaagaacagtacaattcgacctaccgcgtcgtgtccgtgctcacggtgttgcatcaggattggctgaacgggaaggaatacaagtgcaaagtgtccaacaaggcgctgccggcaccgatcgagaaaactatctccaaagcgaagggacagcctagggaacctcaagtctacacgctgccaccatcacgggatgaactgactaagaatcaagtctcactgacttgtctggtgaaggggttttaccctagcgacattgccgtggagtgggaatccaacggccagccagagaacaactacaagactacccctccagtgctcgactcggatggatcgttcttcctttactcgaagctcaccgtggataagtcccggtggcagcagggaaacgtgttctcctgctcggtgatgcatgaagccctccataaccactatacccaaaagtcgctgtccctgtcgccgggaaag

SEQ ID NO: 25 - DNA, 657 bp, Artificial Sequence
  recombinant sequence
gacattgtgatgacccagtcccccgattcgcttgcggtgtccctgggagaacgggccaccattaactgcaagagctcacagtccgtcctgtattcatcgaacaacaagaattacctcgcatggtatcagcagaagcctggacagcctcccaagctgctcatctactgggctagcacccgcgaatccggggtgccggatagattctccggatcgggttcgggcactgacttcactctgactatcaactcactgcaagccgaggatgtcgcggtgtacttctgtcagcagtactacgacaccccgacctttggacaaggcaccagactggagattaagcgtacggtggccgctccctccgtgttcatcttcccaccctccgacgagcagctgaagtccggcaccgcctccgtcgtgtgcctgctgaacaacttctacccccgcgaggccaaggtgcagtggaaggtggacaacgccctgcagtccggcaactcccaggaatccgtcaccgagcaggactccaaggacagcacctactccctgtcctccaccctgaccctgtccaaggccgactacgagaagcacaaggtgtacgcctgcgaagtgacccaccagggcctgtccagccccgtgaccaagtccttcaaccggggcgagtgc

SEQ ID NO: 26 - DNA, 1353 bp, Artificial Sequence
  recombinant sequence
caagtgcaactggtggaatccggggccgaagtgaaaaagcccggagccactgtgaagatctcttgcaaagtgtccggctacaccttcaccgactattacatgcactgggtccagcaggcacctgggaagggccttgagtggatgggtctggtcgatcccgaggacggcgaaactatctacgccgagaagttccagggtcgcgtcaccatcaccgccgacacttccaccgacaccgcgtacatggagctgtccagcttgaggtccgaggacacagccgtgtactactgcgccacggatgctcggggaagcggcagctactacccgaaccacttcgactactggggacagggcactctcgtgactgtctcgagcgcttctacaaagggcccctccgtgttccctctggccccttgctcccggtccacctccgagtctaccgccgctctgggctgcctggtcaaggactacttccccgagcccgtgacagtgtcctggaactctggcgccctgacctccggcgtgcacaccttccctgccgtgctgcagtcctccggcctgtactccctgtcctccgtcgtgaccgtgccctcctccagcctgggcaccaagacctacacctgtaacgtggaccacaagccctccaacaccaaggtggacaagcgggtggaatctaagtacggccctccctgccccccctgccctgcccctgaatttctgggcggaccttccgtgttcctgttccccccaaagcccaaggacaccctgatgatctcccggacccccgaagtgacctgcgtggtggtggacgtgtcccaggaagatcccgaggtccagttcaattggtacgtggacggcgtggaagtgcacaatgccaagaccaagcccagagaggaacagttcaactccacctaccgggtggtgtccgtgctgaccgtgctgcaccaggactggctgaacggcaaagagtacaagtgcaaggtgtccaacaagggcctgccctccagcatcgaaaagaccatctccaaggccaagggccagccccgcgagccccaggtgtacaccctgccccctagccaggaagagatgaccaagaaccaggtgtccctgacctgtctggtcaagggcttctacccctccgacattgccgtggaatgggagtccaacggccagcccgagaacaactacaagaccaccccccctgtgctggacagcgacggctccttcttcctgtactctcggctgaccgtggacaagtcccggtggcaggaaggcaacgtcttctcctgctccgtgatgcacgaggccctgcacaaccactacacccagaagtccctgtccctgagcctgggcaag

SEQ ID NO: 27 - DNA, 657 bp, Artificial Sequence; identical to SEQ ID NO: 25
  recombinant sequence

SEQ ID NO: 28 - protein, 448 aa, Artificial Sequence
  recombinant sequence
QVQLVQSGAEVKKPGATVKISCKVSGYTFTDYYMHWVQQAPGKGLEWMGLVDPEDGETIYAEKFQGRVTITADTSTDTAYMELSSLRSEDTAVYYCATDARGSGSYYPNHFDYWGQGTLVTVSSAKTTPPSVYPLAPGSAAQTNSMVTLGCLVKGYFPEPVTVTWNSGSLSSGVHTFPAVLQSDLYTLSSSVTVPSSTWPSETVTCNVAHPASSTKVDKKIVPRDCGCKPCICTVPEVSSVFIFPPKPKDVLTITLTPKVTCVVVDISKDDPEVQFSWFVDDVEVHTAQTQPREEQFNSTFRSVSELPIMHQDWLNGKEFKCRVNSAAFPAPIEKTISKTKGRPKAPQVYTIPPPKEQMAKDKVSLTCMITDFFPEDITVEWQWNGQPAENYKNTQPIMDTDGSYFVYSKLNVQKSNWEAGNTFTCSVLHEGLHNHHTEKSLSHSPGK

SEQ ID NO: 29 - protein, 219 aa, Artificial Sequence
  recombinant sequence
DIVMTQTPDSLAVSLGERATINCKSSQSVLYSSNNKNYLAWYQQKPGQPPKLLIYWASTRESGVPDRFSGSGSGTDFTLTINSLQAEDVAVYFCQQYYDTPTFGQGTRLEIKRTDAAPTVSIFPPSSEQLTSGGASVVCFLNNFYPKDINVKWKIDGSERQNGVLNSWTDQDSKDSTYSMSSTLTLTKDEYERHNSYTCEATHKTSTSPIVKSFNRNEC

SEQ ID NO: 30 - protein, 454 aa, Artificial Sequence
  recombinant sequence
QVQLVESGAEVKKPGATVKISCKVSGYTFTDYYMHWVQQAPGKGLEWMGLVDPEDGETIYAEKFQGRVTITADTSTDTAYMELSSLRSEDTAVYYCATDARGSGSYYPNHFDYWGQGTLVTVSSASTKGPSVFPLAPSSKSTSGGTAALGCLVKDYFPEPVTVSWNSGALTSGVHTFPAVLQSSGLYSLSSVVTVPSSSLGTQTYICNVNHKPSNTKVDKKVEPKSCDKTHTCPPCPAPELLGGPSVFLFPPKPKDTLMISRTPEVTCVVVDVSHEDPEVKFNWYVDGVEVHNAKTKPREEQYNSTYRVVSVLTVLHQDWLNGKEYKCKVSNKALPAPIEKTISKAKGQPREPQVYTLPPSRDELTKNQVSLTCLVKGFYPSDIAVEWESNGQPENNYKTTPPVLDSDGSFFLYSKLTVDKSRWQQGNVFSCSVMHEALHNHYTQKSLSLSPGK

SEQ ID NO: 31 - protein, 219 aa, Artificial Sequence; identical to SEQ ID NO: 19
  recombinant sequence

SEQ ID NO: 32 - protein, 227 aa, Artificial Sequence
  recombinant sequence
QVQLVQSGAEVKKPGATVKISCKVSGYTFTDYYMHWVQQAPGKGLEWMGLVDPEDGETIYAEKFQGRVTITADTSTDTAYMELSSLRSEDTAVYYCATDARGSGSYYPNHFDYWGQGTLVTVSSASTKGPSVFPLAPSSKSTSGGTAALGCLVKDYFPEPVTVSWNSGALTSGVHTFPAVLQSSGLYSLSSVVTVPSSSLGTQTYICNVNHKPSNTKVDKKVEPKSC

SEQ ID NO: 33 - protein, 219 aa, Artificial Sequence; identical to SEQ ID NO: 17
  recombinant sequence

SEQ ID NO: 34 - protein, 451 aa, Artificial Sequence
  recombinant sequence
QVQLVQSGAEVKKPGATVKISCKVSGYTFTDYYMHWVQQAPGKGLEWMGLVDPEDGETIYAEKFQGRVTITADTSTDTAYMELSSLRSEDTAVYYCATDARGSGSYYPNHFDYWGQGTLVTVSSASTKGPSVFPLAPCSRSTSESTAALGCLVKDYFPEPVTVSWNSGALTSGVHTFPAVLQSSGLYSLSSVVTVPSSSLGTKTYTCNVDHKPSNTKVDKRVESKYGPPCPPCPAPEFLGGPSVFLFPPKPKDTLMISRTPEVTCVVVDVSQEDPEVQFNWYVDGVEVHNAKTKPREEQFNSTYRVVSVLTVLHQDWLNGKEYKCKVSNKGLPSSIEKTISKAKGQPREPQVYTLPPSQEEMTKNQVSLTCLVKGFYPSDIAVEWESNGQPENNYKTTPPVLDSDGSFFLYSRLTVDKSRWQEGNVFSCSVMHEALHNHYTQKSLSLSLGK

SEQ ID NO: 35 - protein, 219 aa, Artificial Sequence; identical to SEQ ID NO: 17
  recombinant sequence